European Patent Application EP 4 292 433 A2, published December 20, 2023. Title: Paenibacillus strains. Applicant: BASF SE. The sequence listing filed with the application follows.

SEQUENCE LISTING (27 sequences)

SEQ ID NO: 1 - DNA, 1539 bp, Paenibacillus sp.
  source 1..1539: mol_type = genomic DNA
  misc_feature 1..1539: note = Unsure note 37,58,60,65,82,87,89,204,263,645,1020,1264,1457; note = Organism note: Paenibacillus polymyxa spp. plantarum; note = Strain Lu16774 complete 16S rDNA
tttgatcctggctcaggacgaacgctggcggcgtgcntaatacatgcaagtcgagcgngnttatntagaagcttgcttctanaattncnagcggcggacgggtgagtaacacgtaggcaacctgcccacaagacagggataactaccggaaacggtagctaatacccgatacatccttttcctgcatgggagaaggaggaaagncggagcaatctgtcacttgtggatgggcctgcggcgcattagctagttggtggggtaanggcctaccaaggcgacgatgcgtagccgacctgagagggtgatcggccacactgggactgagacacggcccagactcctacgggaggcagcagtagggaatcttccgcaatgggcgaaagcctgacggagcaacgccgcgtgagtgatgaaggttttcggatcgtaaagctctgttgccagggaagaacgtcttgtagagtaactgctacaagagtgacggtacctgagaagaaagccccggctaactacgtgccagcagccgcggtaatacgtagggggcaagcgttgtccggaattattgggcgtaaagcgcgcgcaggcggctctttaagtctggtgtttaatcccgaggctcaacttcgggtcgcactggaaactggngagcttgagtgcagaagaggagagtggaattccacgtgtagcggtgaaatgcgtagagatgtggaggaacaccagtggcgaaggcgactctctgggctgtaactgacgctgaggcgcgaaagcgtggggagcaaacaggattagataccctggtagtccacgccgtaaacgatgaatgctaggtgttaggggtttcgatacccttggtgccgaagttaacacattaagcattccgcctggggagtacggtcgcaagactgaaactcaaaggaattgacggggacccgcacaagcagtggagtatgtggtttaattcgaagcaacgcgaagaaccttaccaggtcttgacatccctctgaccggtctagagatagncctttccttcgggacagaggagacaggtggtgcatggttgtcgtcagctcgtgtcgtgagatgttgggttaagtcccgcaacgagcgcaacccttatgcttagttgccagcaggtcaagctgggcactctaagcagactgccggtgacaaaccggaggaaggtggggatgacgtcaaatcatcatgccccttatgacctgggctacacacgtactacaatggccggtacaacgggaagcgaagncgcgaggtggagccaatcctagaaaagccggtctcagttcggattgtaggctgcaactcgcctacatgaagtcggaattgctagtaatcgcggatcagcatgccgcggtgaatacgttcccgggtcttgtacacaccgcccgtcacaccacgagagtttacaacacccgaagtcggtgaggtaaccgcaaggngccagccgccgaaggtggggtagatgattggggtgaagtcgtaacaaggtagccgtatcggaaggtgcggctggatcacctc

SEQ ID NO: 2 - DNA, 1545 bp, Paenibacillus sp.
  source 1..1545: mol_type = genomic DNA
  misc_feature 1..1545: note = Strain Lu17007 complete 16S rDNA; note = Unsure note: 58,60,65,82,87,645,1020; note = Organism note: Paenibacillus polymyxa ssp. plantarum
tttgatcctggctcaggacgaacgctggcggcgtgcctaatacatgcaagtcgagcgngnttatntagaagcttgcttctanataanctagcggcggacgggtgagtaacacgtaggcaacctgcccacaagacagggataactaccggaaacggtagctaatacccgatacatccttttcctgcatgggagaaggaggaaagacggagcaatctgtcacttgtggatgggcctgcggcgcattagctagttggtggggtaawggcctaccaaggcgacgatgcgtagccgacctgagagggtgatcggccacactgggactgagacacggcccagactcctacgggaggcagcagtagggaatcttccgcaatgggcgaaagcctgacggagcaacgccgcgtgagtgatgaaggttttcggatcgtaaagctctgttgccagggaagaacgtcttgtagagtaactgctacaagagtgacggtacctgagaagaaagccccggctaactacgtgccagcagccgcggtaatacgtagggggcaagcgttgtccggaattattgggcgtaaagcgcgcgcaggcggctctttaagtctggtgtttaatcccgaggctcaacttcgggtcgcactggaaactggngagcttgagtgcagaagaggagagtggaattccacgtgtagcggtgaaatgcgtagagatgtggaggaacaccagtggcgaaggcgactctctgggctgtaactgacgctgaggcgcgaaagcgtggggagcaaacaggattagataccctggtagtccacgccgtaaacgatgaatgctaggtgttaggggtttcgatacccttggtgccgaagttaacacattaagcattccgcctggggagtacggtcgcaagactgaaactcaaaggaattgacggggacccgcacaagcagtggagtatgtggtttaattcgaagcaacgcgaagaaccttaccaggtcttgacatccctctgaccggtctagagatagncctttccttcgggacagaggagacaggtggtgcatggttgtcgtcagctcgtgtcgtgagatgttgggttaagtcccgcaacgagcgcaacccttatgcttagttgccagcaggtcaagctgggcactctaagcagactgccggtgacaaaccggaggaaggtggggatgacgtcaaatcatcatgccccttatgacctgggctacacacgtactacaatggccggtacaacgggaagcgaagccgcgaggtggagccaatcctagaaaagccggtctcagttcggattgtaggctgcaactcgcctacatgaagtcggaattgctagtaatcgcggatcagcatgccgcggtgaatacgttcccgggtcttgtacacaccgcccgtcacaccacgagagtttacaacacccgaagtcggtgaggtaaccgcaaggagccagccgccgaaggtggggtagatgattggggtgaagtcgtaacaaggtagccgtatcggaaggtgcggctggatcacctcctttct

SEQ ID NO: 3 - DNA, 1547 bp, Paenibacillus sp.
  source 1..1547: mol_type = genomic DNA
  misc_feature 1..1547: note = Organism note: Paenibacillus epiphyticus; note = Strain Lu17015 complete 16S rDNA; note = Unsure note: 68,87,1024
tgagtttgatcctggctcaggacgaacgctggcggcgtgcctaatacatgcaagtcgagcggggttgnttagaagcttgcttctaancaacctagcggcggacgggtgagtaacacgtaggcaacctgcccacaagacagggataactaccggaaacggtagctaatacccgatacatccttttcctgcatgggagaaggaggaaagacggagcaatctgtcacttgtggatgggcctgcggcgcattagctagttggtggggtaaaggcctaccaaggcgacgatgcgtagccgacctgagagggtgatcggccacactgggactgagacacggcccagactcctacgggaggcagcagtagggaatcttccgcaatgggcgaaagcctgacggagcaacgccgcgtgagtgatgaaggttttcggatcgtaaagctctgttgccagggaagaacgtcttgtagagtaactgctacaagagtgacggtacctgagaagaaagccccggctaactacgtgccagcagccgcggtaatacgtagggggcaagcgttgtccggaattattgggcgtaaagcgcgcgcaggcggctctttaagtctggtgtttaatcccgaggctcaacttcgggtcgcactggaaactggggagcttgagtgcagaagaggagagtggaattccacgtgtagcggtgaaatgcgtagatatgtggaggaacaccagtggcgaaggcgactctctgggctgtaactgacgctgaggcgcgaaagcgtggggagcaaacaggattagataccctggtagtccacgccgtaaacgatgaatgctaggtgttaggggtttcgatacccttggtgccgaagttaacacattaagcattccgcctggggagtacggtcgcaagactgaaactcaaaggaattgacggggacccgcacaagcagtggagtatgtggtttaattcgaagcaacgcgaagaaccttaccaggtcttgacatccctctgaccggtctagagatagncctttccttcgggacagaggagacaggtggtgcatggttgtcgtcagctcgtgtcgtgagatgttgggttaagtcccgcaacgagcgcaacccttatgcttagttgccagcaggtcaagctgggcactctaagcagactgccggtgacaaaccggaggaaggtggggatgacgtcaaatcatcatgccccttatgacctgggctacacacgtactacaatggccggtacaacgggaagcgaaatcgcgaggtggagccaatcctagaaaagccggtctcagttcggattgtaggctgcaactcgcctacatgaagtcggaattgctagtaatcgcggatcagcatgccgcggtgaatacgttcccgggtcttgtacacaccgcccgtcacaccacgagagtttacaacacccgaagtcggtggggtaacccgcaagggagccagccgccgaaggtggggtagatgattggggtgaagtcgtaacaaggtagccgtatcggaaggtgcggctggatcacctcct

SEQ ID NO: 4 - DNA, 1143 bp, Paenibacillus sp.
  source 1..1143: mol_type = genomic DNA
  misc_feature 1..1143: note = Organism note: Paenibacillus polymyxa spp. plantarum; note = Strain Lu16774 dnaN
atgaagattagcattctgaaaaacgttttgaacgaggccatacaacatgtatccaaagcgatatccagtcgaacgacaattccaattttgagtggtattaagctggatgtgaatcaccagggagtcacactgaccgccagcgatacagacatctctattcaatcctttattccgatggaggatggtgaccaaacggtcgttcagatcgaacaacccggcagtgtagtgctacccgctaaattctttgtcgaaattatcaaaaagttgccgtctcaggagatccgtatggaggtaaaagaccaattccaaacctttatctcatccggtgctactgaaattcagatcgttggtttggaccctgaagaatttccggtgcttcccaacattgaagaaaatcaagtgatctctgtgccaggtgatttgcttaaaaatatgattaaacagacggtattctccatctctacccatgaaacgacacctattttgactggtgtattgtggaatctggctgagggcgaattgaaatttgtcgcaacggaccgccaccgccttgccacccgcagcgctcatttggagacgtctgaaggcttgcgttttagcaatgttgtcattgcaggcaaaacgctcaatgagctgagcagaattattccggatcaaaatatgcttgtggatatcgtcgtagcggacaatcaggtattatttaaggtggatcgcgtgttattttactctcgcatcttggacggcacctatcctgatacttctagaattattccgacttcctacaaaacagaactgattgtggacacaaaaagtttgagcgagtctattgaccgtgcttatttgctgtcccgtgaggaaaaaacgaatattgtaaaaatgcaatcgttggaaaacggtgatctagagatttcctccagctcatctgaacttggtaaagtgcgtgaggaagtaaatgtatccaaatttgagggagagccactcaaaatctcgttcaactccaaatatatgctcgacgtgctgaaggtaattgacagcgagcagctgacgattgcttttaccggcattatgagccccattattttaaaaccggcagattccagcaatgcgctgtatatcatcctgccatatcgcacaaccaactag

SEQ ID NO: 5 - DNA, 1980 bp, Paenibacillus sp.
  source 1..1980: mol_type = genomic DNA
  misc_feature 1..1980: note = Organism note: Paenibacillus polymyxa spp. plantarum; note = Strain Lu16774 gyrB
atggtcgacaaaatcgacttgtctgcgggagcttccggtacacagaacggagcttcagaatatggcgcggacgacattcaagtgctcgaagggcttgtggcagttcgcaaacggccgggcatgtacatcgggagcaccagttcttcgggactgcatcatttggtatgggaaattgtagacaacgcggtggatgaacatctcgccaagttttgctctcgcattgatatcacaatgcataaggacggttctgttacagtatcagacaacgggcgcggtattcctacgggaatgcacaaaatgggaattcctacgcctcaagttgtattcaccattttgcacgccggaggtaagtttggcggttcgggatataaaaagtccgggggtctgcatggggtaggtgcgtctgtaacgaacgctctttcggaatggcttgaagtggaaatctaccgggacggcaagattcaccgtcagcggtttgaatattggcaggacaagaagggcgtggagcatgtcggtgaaccgaccacaggccttgaagtgctgggcaatactaacaagacgggctcgaaaattacatttaaaccggatattcgcgtttttcagtcaggaattcattttaactacgatacgctggctgaacgccttcaggagattgcttttctgaattccggccttcgtattcagcttaaagacgaacgcagcggaaagtcagatgaatatttttatgagggtggagcaagtcagtttgtttcttttttgaatgagggtaaggatgtactgcatgatgttattcactttaatgccgagaaagaagacattgaagtggagattgccatccaatacaatgccggctacacagagacgattgcttcgttcgttaactccattccgacacgtggcgggggtacgcatgaaacaggcttcaaaaccgcttacactcgtatcatgaacgactatgcacgcaaaacagcgatgttgaaggaaaaggataaaaacctggaaggtaacgatctgcgtgagggtatgatggctgtaatcagtgtcaagatggccgaggttgaatttgtcggtcagacaaaagatcagctgggtagtgcttcggcgcggagtacagtggatgccatcgtatctgaacaaatgcagcgctttttggaggaaaatccacagatagcgcaaaccttgatcagaaaggcagttcaagcatccaaagcgcgtgaagctgcacgtaaggctcgggacgaaatgcgttctggcaagaaacgcagtgaaagttctaatttgaatggcaaactgtcgcctgcgcagtctaaggattttacacgtaatgagttatttatcgtggaaggcgattcggctggaggatcggccaaacaaggacgggattccaaaatccaggcaattttgccgttaaagggcaagccgatgaatccggaaaaatcaaagttggcggatattatgaaaaatgatgagtatcgtgcgattacggcagcgattggcgcgggggtaggaactgagttcacgctggaagacagcaattattccaaaatcatcattatgaccgatgcagatacagatggcgcgcacattcaagtactgttgttgacgttcttttatcggtacatgaaagaactcattgatgcaggacgcatatttattgctcagccgccattgtataaaataacccgcaagtcgggtaagctcgaaacggttcgttatgcctggactgacgagcagcttgataattacttaaaagaatttggacgaaattttgagcttcaacgttataaaggactcggggagatgaaccctgatcagttatgggaaacgacaatgaatcccgagtcacgcaccctgttgcgcgttcagattgaggatgctgccaaagctgaacgccgtgtgtccacattgatgggtgataaggtggatccacgtaagcgctggatcgtggaaaacgtggatttcacggaatacgtagagtag

SEQ ID NO: 6 - DNA, 1116 bp, Paenibacillus sp.
  source 1..1116: mol_type = genomic DNA
  misc_feature 1..1116: note = Organism note: Paenibacillus polymyxa spp. plantarum; note = Strain Lu16774 recF
gtgtttgtgaacaacattgttttgcagcagtaccggaactataaacagctggagctgaatgaattcgggcccgttaatttgctgatcggacaaaatgcgcaaggcaaaacgaatctggttgaggcgatttttgtattagccttaactaaaagtcaccgaacgtcccgtgacaaggaattaatttctttcggggctacttccacacatctagctgctgatgtggataagaaatacgggaaaatcagattggatctctcgttatccacacaaggcaaaaaagcaaagatcaacgggctagagcagcgaaagctgagcgattttatcggttcgttaaacgtggtcatgtttgcgcccgaggatctggaaattgtcaaaggaacaccgggggttcgccgccggtttcttgacatggaaattggacaagttgcgccaggatatttgtatcatttgcagcaatatcagaaagtgctggttcagcggaataacctgctcaagcaagcttgggggaaagatatggcgtccgtgcagctgatgctggaggtatggaatgagcaacttgttgagcatggtgttaaaattgtaaaaaagcggaaacaatttataacaaagctacaaaagtgggcccaagccattcatgaagggattgcaggtgggacagaagagttaaaattagcctatgttccctctttcggtgagccagaggaagaagatgaagctgtcttattggagcgatttatgataaagttatcccaaatgagggaacaggaaatccgccgtggcatgactttggcgggaccccatcgtgatgatttggcctttgccattaacggcagagaagtgcatacgtatggctctcaggggcagcagcggacgacggccctgtctttgaagctggccgaaatagaattaattcatgaggaaattggggagtatcctatcctgctgctggatgatgtattgtccgagctggacccctatcgtcagactcagctgatcgagactttccaaagcaaggtacagacctttatcacggcaaccgggattgagacgttgaacgcagaacgacttaagggtgcccatatttatcacgtccacgacgggcatgtggaacactaa

SEQ ID NO: 7 - DNA, 1719 bp, Paenibacillus sp.
  source 1..1719: mol_type = genomic DNA
  misc_feature 1..1719: note = Strain Lu16774 recN; note = Organism note: Paenibacillus polymyxa spp. plantarum
atgctggtcactttgtctatacggaatttggcagtcgtagaagctgtcgatgttcatttttataaaggatttcatgtattgagcggagaaactggtgctggtaaatccattattatcgacgcacttgggctgattgcgggcggcaggggatctgctgatctagtgcgttacggatgtgataaagccgaaatggaagccttgtttgaattgccggtcaaacatcccgtttggaatacgttggaggaacaagggattaaggctaatccagaagagcatttgctgattcgtcgagaacttacagttcaggggaaaagctcatctcgaattaacggtcagatggttaatttaacgatgctgcgtgaggtaggtgagcaactcgttaatatccacgggcagcatgagcatcaaagcttgctgcgtgcggatcgccatcttgcgctgctggatacgttcggtgactcggtcattggtccagtcaaagcgctttaccgggagcgctacaatgcttttgtcaaagcggaaaaagaagtaagagaattgcaaagctccagtcaaaaggcttatcagctattggacatgtatcgcttccaattggaagagatcgctgcggcggagttaaaattgggtgaagatgaattattggcagaggaacgggtcaagctatcccatagtgagaaaatgatggatggagtatcaggagcatacgagctgttaagtggcagaggtggtctggatacggtcaataacgtgttgtccagattaaatgatgttcagagctacgacagtaaaagccttcagcccattgcggagcagattcaatctgctttctatcagttggaggatgcagcgtttcaattacgctcttatcgtgaggatattgaatttaatccgggcaagctgcatgaggtggagcaacgtttgaatcaaattaccgggttacagcgaaaatatggtgatagtatagagcagattttggaatactatagccgtattgagcaggaaaccgatctgttggaaaataaagatgagcggctggagcagctcattgcaaagcgggatgagttgctttcgaatttgctggagattgctgaagagcttacagaggcacgtgaaatttgtgctgaagagcttgcagagcaagtagagcaggaattaaaagatcttcaaatggaaagaacgtcactcaaggtgcgtattgatccaattgaagatccacgtggatatgaatataaaggtctaaaggtacgacctaccaagcaagggatagataatgcggaatttctgatttcgcccaatccaggtgagccacttcgcccactcggtaaaatcgcttccggtggtgagttatcacgtatcatgttggcgatgaaaagtatttttgcgcgtcatgatcaaattccggtgctcatttttgacgaggtggataccggggtaagtggtcgtgcagctcagtccatagccgagaagctttatcgtttgtcttccgtttgtcaggtgttttccattactcatttgccgcaggtggcatgtatggcagatcatcagtacctgattgagaaaaatgttcatgacggacggaccatgactcaaattgagggactaacggaggaaggtcgtgttaaggaattggcacggatgctgggtggggtagaaattaccgaaaaaacattgcatcacgcacaggaaatgctgaatttggcggaaggaaagaaagcctga

SEQ ID NO: 8 - DNA, 945 bp, Paenibacillus sp.
  source 1..945: mol_type = genomic DNA
  misc_feature 1..945: note = Organism note: Paenibacillus polymyxa spp. plantarum; note = Strain Lu16774 rpoA
gtgatagaaatcgaaaagccgaaaattgagacggttgacgtcaatgatgatggcacctatggaaaattcgtagtagaaccgctggaacgcggatacggtacgacgcttgggaactcgcttcgccgtattctgttatcctcgttaccgggggcagcagtcacatcggttcagatcgatggggttctgcacgagtttgcaacggttcccggtgtgaaggaagacgtaacggagatcattctgaacttgaaagctttatcgcttaaaatccactcagatgaagagaaagtacttgaaatcgatgcggaaggcgaaggagttgtaacggcaggtgatatccgtgcggatagtgatgtggaaattcttaatccggatcttcacattgcaacgctcggaccgggttcgagacttcacatgcgtatttttgccaatcgcggtcgcggttacgttaagcaggatcggaataaacgtgatgaccagccgatcggcgtcattcccgtcgactccatctacactccgattgcacgcgtgaactacggcgtagaaaatacgcgtgtcggccaggttacgaattatgacaagctgacacttgaggtttggactgacggaactattcgtcctgaagaagctgtgagccttggagccaaaattttgaccgagcatgtgatgctattcgtgggtctcacggatgaagcaaaagatgcagaaattatggtcgaaaaagaagaagacaaaaaagaaaaagttcttgaaatgacgatcgaagagctggatctctccgtccgttcctataactgccttaagcgcgctggtatcaatacggtacaagaactcacgactaaatctgaagaagatatgatgaaggtccgtaacttgggtcgcaaatctttggaagaagtacaagagaagctcgaggaacttggtttaggacttcgtacggaagaatag

SEQ ID NO: 9 - DNA, 1143 bp, Paenibacillus sp.; identical to SEQ ID NO: 4
  source 1..1143: mol_type = genomic DNA
  misc_feature 1..1143: note = Organism note: Paenibacillus polymyxa spp. plantarum; note = Strain Lu17007 dnaN

SEQ ID NO: 10 - DNA, 1980 bp, Paenibacillus sp.; identical to SEQ ID NO: 5
  source 1..1980: mol_type = genomic DNA
  misc_feature 1..1980: note = Strain Lu17007 gyrB; note = Organism note: Paenibacillus polymyxa spp. plantarum

SEQ ID NO: 11 - DNA, 1116 bp, Paenibacillus sp.; identical to SEQ ID NO: 6
  source 1..1116: mol_type = genomic DNA
  misc_feature 1..1116: note = Strain Lu17007 recF; note = Organism note: Paenibacillus polymyxa spp. plantarum

SEQ ID NO: 12 - DNA, 1719 bp, Paenibacillus sp.; identical to SEQ ID NO: 7
  source 1..1719: mol_type = genomic DNA
  misc_feature 1..1719: note = Organism note: Paenibacillus polymyxa spp. plantarum; note = Strain Lu17007 recN

SEQ ID NO: 13 - DNA, 945 bp, Paenibacillus sp.; identical to SEQ ID NO: 8
  source 1..945: mol_type = genomic DNA
  misc_feature 1..945: note = Organism note: Paenibacillus polymyxa spp. plantarum; note = Strain Lu17007 rpoA

SEQ ID NO: 14 - DNA, 1143 bp, Paenibacillus sp.
  source 1..1143: mol_type = genomic DNA
  misc_feature 1..1143: note = Strain Lu17015 dnaN; note = Organism note: Paenibacillus epiphyticus
atgaagatcagcattctgaaaaacgttttgaacgaggctatacaacatgtatccaaagcgatatcaagtcggactacgattccaattctgagtggtattaagctggatgtgaatcaccagggagtaacgctgaccgccagcgatacagacatctccattcaatcctttattccgatggaggatggtgaccaaactgttgttcaggtcgaacaacccggcagtgttgtgctgcctgccaaattctttgtcgaaattatcaaaaagttgccgtcgcaggagatccatatggaggtaaaagaccaatttcaaacctttatctcgtctggcgcaactgaaattcagattgttggcttggaccctgaagaattcccggtgcttcccaacattgaagaaaatcaagtcatctctgtaccaggagatttacttaaaaatatgattaaacagacggtattctccatctccacccacgaaacgacaccgattttaactggcgtgttgtggaatctggctgagggtgaattgaagtttgtggcaacggaccgccaccgccttgccacccgtagcgctcatttggagacgtctgaaggcttgcgttttagcaatgttgtcattgcgggcaaaacgctgaatgagctgagcagaattattccagatcaaaatatgcttgtggatatcgtagtagcggacaatcaggtattattcaaagtagatcgggtgctattttattcccgcatcttggacggcacctatcctgatacttctagaattattccgacctcctacaaaacagaactgattgtggatacaaaaagtttaagtgagtcaattgaccgtgcttatttgctgtcccgtgaggaaaaaacgaatattgtaaaaatgcagtcgctggaaaatggcggtttggagatttcctctagttcctctgagcttggcaaagtgcgtgaggaagtaactgtgtccaaatttgagggagagccgctcaaaatttcgttcaactctaaatacatgctcgacgtgctgaaggtgattgacagcgagcagctgacgattgcttttaccggcattatgagccccattattttaaaaccggctgattccagcaatgcgctgtatatcatcctgccatatcgcacaaccaactga

SEQ ID NO: 15 - DNA, 1980 bp, Paenibacillus sp.
  source 1..1980: mol_type = genomic DNA
  misc_feature 1..1980: note = Strain Lu17015 gyrB; note = Organism note: Paenibacillus epiphyticus
atggtcgacaaaatcgacttgtctgcgggagtgtccggcacacaaagcggagcttcggaatatggcgcggacgacattcaagtgctcgaagggcttgtggcagttcgcaaacggccgggcatgtacatcgggagcaccagttcttcggggctgcatcatttggtatgggaaattgtagacaacgcggtggatgaacatctcgccaagttttgctctcgcattgatattacaatgcataaggacggttccgttacagtatcagacaacgggcgcggtattcctacgggaatgcacaaaacgggaattcctacgcctcaggttgtattcaccattttgcacgccggaggtaagtttggcggttcgggatataaaaaatccgggggtctgcacggtgtaggtgcgtctgtaacgaacgctctttcggaatggcttgaagtagaaatttaccgggacggcaagattcaccgtcagcggtttgaatattggcaggacaagaagggcgtggagcatgtcggggaaccgaccacaggccttgaagtgctgggcaatactaacaagacgggctcgaaaattacatttaaaccggatattcgtgtttttcaggcaggcattcattttaactacgatacgttggctgagcgccttcaggaaattgcttttctaaattcgggccttcgtattcaacttaaagacgaacgcagcggaaagtcagatgagtatttttatgagggtggcgcaagtcagtttgttgcttttctgaatgagggcaaggatgtgctgcatgacgttattcactttaatgccgagaaagaagacattgaagtagagattgccatccagtacaatgctggttatacagagacgattgcttcgttcgttaactccattccgacacgtggaggaggtacgcatgaaacgggattcaaaaccgcttacactcgtgtcatgaacgactatgcccggaaaacggtgatgttgaaagaaaaggataaaaacttggagggcaacgatctacgtgagggcatgatggctgtaatcagtgtcaagatggctgaggttgaatttgtcggccagacaaaggatcagctgggaagcgcttcggcacggagtacagtggatgccatcgtatctgagcagatgcagcgttttttggaagaaaatccgcagatagcacaaactttgatcaagaaggcagttcaagcatccagagcacgtgaagctgcacgtaaagctcgggatgaaatgcgttccggtaaaaagcgcagtgaaagttccaatttgaatggtaaactatcgcctgcgcagtccaaggattttacacgtaatgagttgtttattgtggaaggcgattcggctggaggatcagccaagcagggacgggattccaaaattcaggccatattgccgctaaagggcaagccgatgaatccggaaaaatccaaactggcggatattatgaagaatgatgagtaccgtgctattacagcagctattggtgcgggagtaggaacagagttttcgctggaagacagcaattattccaaaatcatcattatgaccgatgcagatacagatggtgcgcacattcaagtgctgttgttgacgttcttttatcggtacatgaaagagcttattgatgcaggacgcatatttattgctcaaccgccattgtataaaataactcgaaagtcgggtaagctcgaaacggtgcgttatgcttggactgacgagcagcttgataattatttaaaagaatttggacgaaattttgagcttcagcgctataaaggacttggggaaatgaaccctgatcagttatgggaaacaacgatgaatcccgattcacgcaccttgctacgcgttcagatagaggatgcagccaaggctgaacgcagggtgtccactttgatgggtgataaggtggatccgcgcaagcgctggatcgtggaaaacgtagattttacggaatacgtagagtag

SEQ ID NO: 16 - DNA, 1116 bp, Paenibacillus sp.
  source 1..1116: mol_type = genomic DNA
  misc_feature 1..1116: note = Strain Lu17015 recF; note = Organism note: Paenibacillus epiphyticus
gtgtttgtgaacaacattgttttgcagcagtaccggaactatgaacagctggagctgaatgaatttgggcccgttaatttgctgatcggacaaaatgcgcagggcaaaacgaatctggtagaggcaatttttgtactggctttaaccaaaagtcatcgaacgtcccgcgacaaggagttaatctctttcggggctacttccactcacctagctgcggatgtggataaaaaatacgggaaaatcagactggatctcgcgttatccacacaaggcaaaaaagcaaagatcaacggactggagcagcgcaaactgagcgattttatcggttcgttaaatgtggtcatgtttgcacctgaggatctggaaattgtgaaaggaacaccgggggttcgccgccggtttcttgacatggaaatcggacaggttgcgccaggatatctgtatcatttgcagcaatatcagaaagtattggttcagcgaaacaacctgctcaagcaagcttggggtaaggatatggcgtcagtgcagctgatgctggaggtatggaatgagcaacttgttgagcatggtgttaaaattgttaaaaagcggaaacaatttataacaaagctacaaaagtgggctcaggccattcatgaagggatcgcaggtgggacagaagagttaaaattaacctatgttccctccttcagtgagccagaggaagaagatgaagctgtcttattggagcgatttatgataaagttatcccaaatgagggaacaggaaatccgccgtggcatgactttggcgggaccccatcgtgacgatttggcctttgccattaacggcagagaagtgcatacgtatggctctcaggggcagcagcggacgacggccctgtccttgaagttggccgaaatagagttaattcatgaggaaattggtgaatatcctgtcttgctgctggatgatgttttgtccgagctggacccctatcgtcagacccagctgatcgagactttccaaagcaaggtacagacctttatcacggcaaccggggttgagactttgaacgcagaacgactcaaggatgccaatatttatcacgtccacgacgggcatgtggaacactaa

SEQ ID NO: 17 - DNA, 1719 bp, Paenibacillus sp.
  source 1..1719: mol_type = genomic DNA
  misc_feature 1..1719: note = Strain Lu17015 recN; note = Organism note: Paenibacillus epiphyticus
atgctggtcactttgtctatacggaatttggcggtcgtagaggccgtcgatgttcatttttataaagggtttcatgtcttgagcggggaaacaggtgctggtaaatccattattatcgatgcgcttggcctgattgcaggcggtaggggctctgctgatctagtgcgttacggttgtgataaagcagagatggaagccttgtttgagctgccggtaaaacatccagtttggaaaacacttgaggaacaagggattaaggccaatgcggaggagcatttgctgattcgtcgcgaacttacggttcaggggaaaagctcttctcgaattaacggtcagatggttaatttaacgatgctgcgtgaggtaggtgagcagctcgtcaatatccacgggcaacatgagcatcaaagcctgctacgtgcagatcgccatctggcgctgctggatacgttcggtgattcggtgatcggtccagtcaaaacgctttaccgtgagcgttacaatgcttttgtcaaagcggaaaaagaagtaagagaactgcaaagctccagtcaaaaggcttatcagcttttggatatgtaccgatttcaattagaagagatcgctgcggcggagttgaaattgggagaagatgaattattggcagaggaacgggtcaagctatcccatagtgagaaaatgatggatgggatatcaggagcatacgaactgctaagcggcagaggtgggctggatacgatcaataacgtattgtctagattgaacgatgtccaaagctatgacagcaaaagccttcagcccattgcggagcagattcagtctgctttttaccagttagaggacgcagcattccaattacgttcttatcgtgaggatattgaatttaatccaggcaagctgcatgaagtggagcaacgtttgaatcaaattaccggattacagcgaaaatatggtgatagtatagagcagattttggaatactatagccgtattgagcaggaaaccgatctgctggaaaataaagatgagcggctggagcagctcattgcaaaacgggatgagttgctttccgatttgctggagatttcagaagagcttacagaagcacgtgaaatttgtgctgaagagcttgcagagcaagtggagcaggagttaaaagacctgcagatggaaagaacgtcactcaaggtgcgcattgatccaattgaagatccacgcggatatgagtataaaggtctgaaggtaaggcctaccaagcaaggaattgataatgcggaatttcttatttcacccaatccaggtgagccactacgtccacttggtaagatcgcttcaggcggtgagctatcacgtatcatgttggcgatgaaaagtatttttgcgcgtcatgatcaaattccagtactcatttttgacgaggtggataccggggtgagtggtcgtgcagctcaatccattgccgagaagctatatcgtttatcttccgtttgtcaggtgttttccattactcatttgccacaggtggcatgtatggcagatcatcagtaccttattgagaaaaatgttcatgatggacggaccatgactcaaattgagggacttacggaggacgggcgtgtcaaggaattggcacggatgctgggcggcgtggaaattaccgaaaaaacattgcatcacgcacaggaaatgctgaatttggcggaaggaaagaaagcctga

SEQ ID NO: 18 - DNA, 945 bp, Paenibacillus sp.
  source 1..945: mol_type = genomic DNA
  misc_feature 1..945: note = Strain Lu17015 rpoA; note = Organism note: Paenibacillus epiphyticus
gtgatagaaatcgaaaagccgaaaattgagacggttgacgtcaatgatgatggcacctatggaaaattcgtagtagaaccgctggaacgcggatacggtacgacgttgggaaactcgcttcgccgtattctgttatcctcgttaccgggggcagcagtcacatcggttcagatcgatggggttctgcacgagtttgcaacggttcccggtgtgaaggaagacgtaacggagatcattctgaacttgaaagctttatcgcttaaaatccactcggatgaagagaaagtactcgaaatcgatgcggaaggcgaaggagttgtaacggcaggagatatccgtgcggatagtgatgtggaaattcttaatccggatcttcacattgctacgctcggaccgggttcgagacttcacatgcgtatttttgccaatcgcggtcgcggttacgttaagcaggatcggaacaaacgtgatgaccagccgatcggcgtcattcccgtcgactccatctacactccgattgcacgcgtgaactacggcgtagaaaatacgcgtgtcggccaggttacgaattacgacaagctgacacttgaggtttggactgacggaagtattcgtcccgaggaagcagtgagccttggagccaaaattttgaccgagcatgtgatgttgttcgtgggtctcacggacgaggcaaaagatgctgaaattatggttgaaaaagaagaagacaagaaagaaaaagttcttgaaatgacgatcgaagagctggatctctccgtccgttcctataactgccttaagcgcgctggtatcaatacggtacaagaactcacgactaaatctgaagaagatatgatgaaggtccgtaacttgggtcgcaaatctttggaagaagtacaagagaagctcgaggaacttggtttaggacttcgtacggaagaatag

SEQ ID NO: 19 - protein, 6 aa, Paenibacillus sp.
  REGION 1..6: note = Compound 1A
  SITE 1..6: note = Cyclic peptide: the hydroxyl group of the side chain of residue position 1 is forming an ester with the carboxy terminus of residue position 6
  SITE 1: note = The amino terminus is forming an ester with 15-guanidino-3-hydroxypentadecanoic acid (GHPD)
  SITE 1..6: note = The stereo configuration of the amino acids of the cyclic peptide has not been elucidated
TIYTNA

SEQ ID NO: 20 - protein, 6 aa, Paenibacillus sp.
  REGION 1..6: note = Compound 1B
  SITE 1..6: note = Cyclic peptide: the hydroxyl group of the side chain of residue position 1 is forming an ester with the carboxy terminus of residue position 6
  SITE 1: note = The amino terminus is forming an ester with 15-guanidino-3-hydroxypentadecanoic acid (GHPD)
  SITE 1..6: note = The stereo configuration of the amino acids of the cyclic peptide has not been elucidated
TIYTQA

SEQ ID NO: 21 - protein, 6 aa, Paenibacillus sp.
  REGION 1..6: note = Compound 2A (fusaricidin C) (LI-F03a)
  SITE 1..6: note = Cyclic peptide: the hydroxyl group of the side chain of residue position 1 is forming an ester with the carboxy terminus of residue position 6
  SITE 1: note = The amino terminus is forming an ester with 15-guanidino-3-hydroxypentadecanoic acid (GHPD)
  SITE 2: note = V is D-Valine
  SITE 4: note = T is D-allo-Threonine
  SITE 5: note = N is D-Asparagine
  SITE 6: note = A is D-Alanine
TVYTNA

SEQ ID NO: 22 - protein, 6 aa, Paenibacillus sp.
  REGION 1..6: note = Compound 2B (fusaricidin D) (LI-F03b)
  SITE 1..6: note = Cyclic peptide: the hydroxyl group of the side chain of residue position 1 is forming an ester with the carboxy terminus of residue position 6
  SITE 1: note = The amino terminus is forming an ester with 15-guanidino-3-hydroxypentadecanoic acid (GHPD)
  SITE 2: note = V is D-Valine
  SITE 4: note = T is D-allo-Threonine
  SITE 5: note = Q is D-Glutamine
  SITE 6: note = A is D-Alanine
TVYTQA

SEQ ID NO: 23 - protein, 6 aa, Paenibacillus sp.
  REGION 1..6: note = Compound 3 (LI-F08b)
  SITE 1..6: note = Cyclic peptide: the hydroxyl group of the side chain of residue position 1 is forming an ester with the carboxy terminus of residue position 6
  SITE 1: note = The amino terminus is forming an ester with 15-guanidino-3-hydroxypentadecanoic acid (GHPD)
  SITE 2: note = I is D-Isoleucine
  SITE 3: note = I is L-allo-Isoleucine
  SITE 4: note = T is D-allo-Threonine
  SITE 5: note = Q is D-Glutamine
  SITE 6: note = A is D-Alanine
TIITQA

SEQ ID NO: 24 - protein, 6 aa, Paenibacillus sp.
  REGION 1..6: note = Compound 4A (LI-F06a)
  SITE 1..6: note = Cyclic peptide: the hydroxyl group of the side chain of residue position 1 is forming an ester with the carboxy terminus of residue position 6
  SITE 1: note = The amino terminus is forming an ester with 15-guanidino-3-hydroxypentadecanoic acid (GHPD)
  SITE 2: note = I is D-allo-Isoleucine
  SITE 4: note = T is D-allo-Threonine
  SITE 5: note = N is D-Asparagine
  SITE 6: note = A is D-Alanine
TIVTNA

SEQ ID NO: 25 - protein, 6 aa, Paenibacillus sp.
  REGION 1..6: note = Compound 4B (LI-F06b)
  SITE 1..6: note = Cyclic peptide: the hydroxyl group of the side chain of residue position 1 is forming an ester with the carboxy terminus of residue position 6
  SITE 1: note = The amino terminus is forming an ester with 15-guanidino-3-hydroxypentadecanoic acid (GHPD)
  SITE 2: note = I is D-allo-Isoleucine
  SITE 4: note = T is D-allo-Threonine
  SITE 5: note = Q is D-Glutamine
  SITE 6: note = A is D-Alanine
TIVTQA

SEQ ID NO: 26 - protein, 6 aa, Paenibacillus sp.
  REGION 1..6: note = Compound 5A (fusaricidin A) (LI-F04a)
  SITE 1..6: note = Cyclic peptide: the hydroxyl group of the side chain of residue position 1 is forming an ester with the carboxy terminus of residue position 6
  SITE 1: note = The amino terminus is forming an ester with 15-guanidino-3-hydroxypentadecanoic acid (GHPD)
  SITE 2: note = V is D-Valine
  SITE 4: note = T is D-allo-Threonine
  SITE 5: note = N is D-Asparagine
  SITE 6: note = A is D-Alanine
TVVTNA

SEQ ID NO: 27 - protein, 6 aa, Paenibacillus sp.
  REGION 1..6: note = Compound 5B (fusaricidin B) (LI-F04b)
  SITE 1..6: note = Cyclic peptide: the hydroxyl group of the side chain of residue position 1 is forming an ester with the carboxy terminus of residue position 6
  SITE 1: note = The amino terminus is forming an ester with 15-guanidino-3-hydroxypentadecanoic acid (GHPD)
  SITE 2: note = V is D-Valine
  SITE 4: note = T is D-allo-Threonine
  SITE 5: note = Q is D-Glutamine
  SITE 6: note = A is D-Alanine
TVVTQA